European Patent Specification EP 3 122 877 B1, published March 22, 2023. Title: TARGETED GENOME EDITING IN ZYGOTES OF DOMESTIC LARGE ANIMALS. Applicant: University of Maryland, College Park. The sequence listing filed with the application follows.

SEQUENCE LISTING (17 sequences)

SEQ ID NO: 1 - DNA, 10988 bp, Sus scrofa
  misc_feature (718)..(817): n is a, c, g, or t
  misc_feature (2967)..(2968): n is a, c, g, or t
  misc_feature (2993)..(2993): n is a, c, g, or t
acgtacgcggccaaaagagtctcaactccctcccagagactcagatttccgaccagcttggcagatcccgggcgccggagcgccagagcgcgcgcgcgcgccgccgccgcctcccttccccgcccgcgcgcctcgccacccctcggcgccagacactgacagccccggagctgcgagcgtcttctgttccagcggtggcaggtaaacagccgggtcgccccgagaactgggggtgccaaggtcgggagtcagaaccccccgccttggagcttaggcgcaagggtgagcggcccacttggggcgctagggaaaccttgacagagaggggggcgggggacttccggcgggcggggggcgcgacaggcctgcccccgcttgttcgtcggcttaacattggccccgctcacatttgctttccaggtggggtgagggccctttactcggaatggggcttggtgggggaagggggtgcctggggctggccgcgacccctgggcagggaggcggatggtggcggggagtctagccctctcccacgcgcgtccgcggctggcggaggatgggagaggcgcgccggcaccggggccgcagggccgggaactcaaggagggtcgcccacggcctccgctgaggcgctcggaggagaaccagggagaggggccggcgtgcggctctcccgaggccccaggggcacgtggggtggggatgatggccccgnnnnnnnnnnnnnnnnnnnnnnnnnnnnnnnnnnnnnnnnnnnnnnnnnnnnnnnnnnnnnnnnnnnnnnnnnnnnnnnnnnnnnnnnnnnnnnnnnnnnagccccaaggggcccgttgggggggggtgatggcccaggccccggcgggaggggcccttgccgccgccaccatggagctcctccggagagacggcccacctgccatccacgcggcccgggggtgctggggaggccgcagcggggtgggcctcctgcatccctggggatggagaccgggcacgtggtccgaccttcgggcctcggcgggcggagtctcgggcggccccaccctcactgtcggccgagacgtccaggtccctgggggccgagtgtccggagagcccaggtgctttgcttttcactgtctccactgcccctccccgaagggaactgggcggtcagaggctcctctcaaggggatcagggccggacagctctcctcctgatccacttgtgtgggctgccctttcaggcttgattgtaaacaacgaggagaagtccatttttactgtcccttttcatttttttcccttttctaaatttgtagcaaccatggcaaatcagtttttaaaatcataacccacagccatcaatccacccttaccatctcaaagccactgctttctgtttttcagttttctgtctccagattcgtacataacgcaaagaaatttcaactgccctgattatgattatcctcctctaatggccgagttattttcttctgcttaaagcgtcgcagtttaataagcagttccccgaatgctgaacatttgaaatgtttcgttttttcttgcaaaaaaaccttccaggtataacagtattaaagaaagaataggaataggagttccctggtggcctggtggttaaggatcccatattgtcgctgctgtggctagagttccatccctggcccggaaacttctgtatacctcaggcaagccaacaaaaagaaaaaaagaagggaagaaaagaaaaaaatagtaacagaaaattgaattaaaatgtcaaacccctggaaaaattaacaactatctcagatttgaggaagaaaaaaaaaatcaacagttttacctgcagtaaacactgaggcgctcttacaatgaaaaagaactaaccggaaagggaaagaaagcagagctaggatgtgatttgtatatgatttgtatctgacacaaaattttcatagttatgaaaggaaaatatgaaaattataataaatgatgaatcaattatagaataaaatgtaaattaaagcactctggattatcattttacaattactaacaaatacaacaacagtaatagtaacagcaaccactgttggaagattgcctagaaattttcacattcagttattttgagaggtggcaggactttggggttagaagaatggctctgcacctaatttcatagcatggaatgggttacctaatttcctcatcctccttttgtgcattcataaaatagaggaaattatacctacttcaggaaattgctaagattaaccatctatgtaaaactgacctttggtatgtaatcctttttctattcttgggcacactgcactggggacattgtgaatttactgtaaagcaatttggtaatgcattaggccatgacccagaatttacctgcaatggaagaaacaacaagaaaaaaaagggggggaaaaaaaagccatatgcagtcacagaattcagaatgatctaaaattagacccaacggaaaaacaacctaaatgtataacagcagggcagcagctgaggaaatcatggctctttaactgaaagaaacattatgtaactatcaaaagtcggtggtacatgagaaaaaactgataaatcagtgtagattacattaccaaactgtatctacttactcagtgaatgcatatgtggaaaatctgaaaggaaaagcatacaaaggaattgaatagaattaaaatgaagttagaaattatgggtcagtttaattttcttttttatttatatactgcttttctaagtaacgaaatttttaagataattattcatcgttctcaatttttgtaatgaaatggagccatagttttctgtatgtgggagagggagagctcagtgtcatgttagctgacttcatttcttcagatattgtctctttttttttctcgtgtagatggattagggggttagtaatgtatatattaggatccttctttaaggaatagnntctaaaaattattatcaattctagntttttctttttttggtgtttctaaggaccctgaatatatttgaaaactgaacagtttcagctaagccgaagcattctgtcttccccagaacacaaatccagcctcgctgagccattacagatgtacatactgcagagtccctttgatctcgtgatggctcagagtccctatctgtcacagaaaagaagggcctagaaaggctatgatgacagtccttgctctgaggcaacttagggttatatgtgtaacccacacctcttaaatcatcctttcttgtaaaatcattttgattttgcaggcaaagggccacggatttctttagaatcactctgagttatacaaggaatcaaccatttaaaaaatacaataaaaaagcaattacaaatatttctgtaccagattaacactgaaggtgactatcagccaacaaaaggttgacagtttttctaagctgtggttttagtttacctattccattctcccttttcagttcttatttcctattccaagacaactgtatatcagctgtgaactgctgcatgtgaaacattcaaaacatgcctctacataaagtggtggctgctgcagaagaatctgagtggatagcatatatagcagttcttacagtgggagtatttttttctcaatttgttcatcctttttcttctaactatattctgcttattgctgttccagtattgtgtgatcacatcaagggaggggtaccctgttatgctttataagtgttaagttttgtgctcctgggacctagctctgaagcctggctaggagtgcagttctctgggaagctttcctgtctttcctgagctaaggtggaactcagcagtcatattttcatcttttgaagtcattgtcccttaaagaatctaatgcaagctatataaaatttttacaaaccattctggggtggggggttttcactggcactctgagacttagccctcgactgaatagggcaaggggcccccaacctggccatcctcagaaataggtgaagagcttttaaaaatgtaacattgctagaacctatcccaggctgacagccaggtgttttctagtgatgggatttaggaatctatattgtagcaggatttaacagtatctgataacagtatattctctcttctttcctcttcctttttaaagttgagtttgttatttgtacacattccttaccccttatggttttattgaactcaaaaaaattgagctggagttttgtcattttattgagattataaattcacttaggggtaactgacatctttagaatactaaattgttccaaccaagactttcccatttttatgggtcattttctttttttttctttttttttttttaattttttttttttttttttttttttttggcctttttttgtcttttgttgttgttgctatttcttggaccgctcccgcggcatatggaggttcccaggctaggggtcgaatcggagctgtagccaccggcctacgccagagccacagcaacggtggatccgagccgcgtctgcaacctacaccacagctcacggcaacgccggatcgttaacccactgagcaagggcagggactgaacccgcaacctcatggttcctagtcggattcgttaaccactgcgccacgacgggaactcctttatgggtcattttctatcttctttattaatgtttaaattttttccccagtcttaatttctcttaagtcagtcctagttacattacagttctggttgaaattatggctattttattaatttttttcctagttgattattgctgctgtagagaaatgctattgatttttataggccaatcttgtatcccacaaccttgccaaactctagtactgagtctagtactgaagtccccttgtggcgcagggggttaaggatcaggcattgcaagcagctgtggtgcaggctgcaattgcagagtggtttcaatccctggcccagaaacttccacatgccacaagtacagccaaaacaaacaaacaaacaaacaaaaacttgtgtcaggtctgttgaattttttatgtatatgatcatccaaattccaaatagtgacagctggagctctttccttgcagttcttgcaccagttacttcgttgcttacagcgttggaaggacctccagtcccatgacagttggcatccttgtcttgcttctgattttaaagggactgcattccaaagttatctattaagtactgttttgtggtataatctttatcaagttaaggaaattccctcctattcctggtctactaaaagtattttttttagtgataaatagatattgacctttatcaaatacttaatgttttaaaatgtatcagaggattaggccacagaatgactgttcaggagtatcttatatgaaatgttataacacagccaggcattcagaaacccagtctccattcccagcaatctcactaattagcattttaatcgcagatatgtcacttgacttagctgaatcttggtggcctaatttgtagagtgcgagattgggattaaataatacaaggtctttcttattttatcacaaacagagattttccatggtctcattaagttttgagtcttcctggagttgcggctgtggctcagtggtagtgaacctgacgggtatccatgaggacatggttcaatccctggccttctcagtgggttaagaatccagccttgctgtgagctgtgatgtaggtcacagaagtggcttggatcctgcgttgctgtggctgtggtataggccagcagctgtagttcctatttgactcctagccagggaattactatatgctgcaggtggggcccaagttttgagtcttccgtatccttagaaatgagtctctccttcaaaatgtagttgttatttttttatgcttttcataagtagatgttgcttttgtcattctcaactggttttaaaacgatcctgtcttaatatagtctatgattatccagctttacctagtattcagtgtttaagtactaatggcaacatatgcctgctccccttacacactgttgcctgtatctccagaccctgttcattcctcagctccagattccccaagctaactgcctacttgtctctcttgtcccacatgcagctggaggatcgcattgccaaagccacacccctcatttgtctccctccaaatttgctccaccttctgtgttctgtctactcaattgcccgatctggaaacttgggtaccacctcgattcttccatactcttactttccacatcaaactgcaagccttccagaaggtgctaatccaccttgttcaggcccctgaggtgttggaacagaattgtgagcagtatggaggcgaagagttgagccccatcagcaaatggatcctggttaggttcattaaccgctaagccatgaagggaactccctaattggcatattttgagcagtttgtgctgataatgttcaaataaatttttatttacaccaagacctttcaaaaggtgtttcttggtgacctagcaggttaaggatccagggttgtaactgctatggctcgggtcagtgctgtagcatgggtgagcttgatccctggctctgggacttcagcatgccatgcgtgcagccaaaaaaaaaaaaaaatttttttaataaatgatagtagaaacaaatgaaatattaactactttatttctttaatcattcttcctctgaatattatacaatttaatctttaactctgaaggttatgaaaaataattttatatttgatgccacttttatttgaagataccctggtgctggggataaaactagtatcagggttatagcatgtgccgtttttggttttatggcacatggtgttttggagtagtacatggtttgacatgaggtccagtagagtctgtttaatggtcattctattctgtgtctttaatcactgcccttggaacccagcacccagggtaaatgacatcttcagtctgaaaggatgtttaatttgatgaatgtacattgtttattcttaagttattctagcccttttatgtcttaatatgtgtcttttgcaccaaaaattaggaggaagtaactcactcatgaactaccgaatgccaaactaaaacttattcagtgactgagtgactgtaaatcttgtgaacacagactttctttttttttttattaaaaatgttctttttaaaaaaattttttttggccaaccactcatggcatgtttgatcaggccagggatcaaacctgaggcagaggcgtaaccagagccacagcagtgacaatgctgaatccttaacctgctgagccaccggggaactcctgaatgcagcctttcttaccccattttgagcagcctcatttgtctgcctatagaaagaaagatgaatttatagatgggcttgcaaaatcttgcatgttttctgtttccaaaaactgttgagaattcctttgaggaaattattgtaggtatttatatattcagaggatattaatttctttacttaatagatacttattgtgtacctgccctataccaggcactgcccaagcccctgaggatatagcagcaaacaaaagagactcattccctgcttacattcccactcaaggaagaaggacacaagtcagctatttaaaaattatttcatgatctcaacacctacctgggggcttcacttccagaggggcctgccaggtccctcaaggtagtccacacagcagttagggccttggcttcactcccagccccagcccccacaagtgaccgctcaggtacaaaggaatgagtctgtgcgtagagggttccccttggcacaggggccctaggccccataggtgctgatagccctcattatagccccattagcagagctgccagggtccctacaagaaggtgcctggttacaagaattattactttacttatttatgcaccatgtggaagtttccaggctagaagtcgaatcagagatgtagctgctggcctacgccacagccataccagatctgagctgcatctgcgacctcaccacagcacacggcaaggccagggatcgaacccgcgtcctcatggatactaatccatggctggtttctgctgagtcatgatgggaactcccagaatcacaaaagctcaaagctgtggcaaacccaccaggtgtttattggtttttccagtttagatacaatgtatcaagcagaggttatttttaccataagcatgttgctggcattccacctttatcttttctaagaaacagagccagaaaattatctgaaggtcaaatttgtccttagagaaggagaaagagttgagttaacccttcacctacagttgtttttgttgtaagtgttgcacaggagacaaatggagtataaagaacattcacagctgatgccgctactatgttcattatgctgcagacattaagtgatttcaatataaacaggacactgacaccctctttattttgtattttgcagataagtaatcatggtgaaaagccatataggtggctggatcctcgttctctttgtggccgcatggagtgacatagggctctgcaagaagcgaccaaagcctggcggaggatggaacactggggggagccgatacccagggcagggtagtcctggaggcaaccgctatccaccccagggagggggtggctggggacagccccacggaggtggctggggacagccccacggaggcggctggggacagccccacggtggcggctggggacagccccatggtggcggaggctggggtcaaggtggtggctcccacggtcagtggaacaagcccagtaagccgaaaaccaacatgaagcatgtggcaggcgccgctgcagctggggcagtggtagggggcctcggcggttacatgctggggagtgccatgagcagacccctgatacactttggcagtgactatgaggaccgttactatcgtgaaaacatgtaccgttaccccaaccaagtgtactacaggccagtggatcagtacagcaaccagaacagttttgtgcatgactgcgtcaacatcaccgtcaagcagcacacagtgaccacgaccaccaagggggagaacttcaccgagacggacgtcaagatgatagagcgcgtggtggaacagatgtgcatcacccagtaccagaaagagtacgaggcgtacgcccaaagaggggccagtgtgatcctcttctcctcccctcctgtgatcctcctcatctctttcctccttttcctcatagtgggctgagggtggcctttctgtcggcatcatcttcttaatctttatcaggttgggggagggaatatctacctgcagccctttagtggtggtgtctcattcttgcttctctcttcggcacccataggctaacatccatggcgcttgtagcactggaaaaggagagtagacctgagatgtgatgtatttaagccccatttgattgaatccttcataggccagtgctagtgctggactggtaagagcgtaacagcaaataatcattggttgatctgggctcattttttgtctggtgcaacagattgaggctaaaacaattctcaaaacacacttcaagtacctttacctaaatacctccagctccttctccagctagagctcagtacacaaatgccccgccatagtagtgattttgtagcaactttcccatttaagaaaacctgactacattttcctgttcaaatagcatttctactgagttggggaggaggccacataatactcattcaaaaaaatgaaactggaaatccttagctcctgggcccagggtcagcccagtggaaagcatgtgtcctgtgtctgcagagaactaaggatattttgcaatttgcagtacaggttacacagcagctattgcatcaagaatggatgtctgtgcaacactagacttctgggcagagggcattttcacaggcaatgaacataactcacataatatgaaaggctctgaaacttaaaaaattcccacctgtgtgaggaaccctcagaggcagccttctgttatggatgtttaaagcaccttcatggggtagttctttctttagtaatacaaactatagataattaaggtagtaggacatgaaacaatcttctggacattgagaacaaatctcttttgtttgtttatctgggaactggagtgattttgccatttcttggatgaagccaggagattttaacatagaggaagctgcagctataaaaacatcatatttattcatttgattgagtctttcatgggccagtgccggtgttgggctagcaagcatatgataccaaatatagagggttatgaagaaaatgattagtgtacaaaaaagagaaatgcttacatttctttattgctgtgtcataattgtcaaaaatcagaattaggtcctcaatttctataattggcttttgaatcaaagaataggaaggcattcccccccaaaaaagttaaagatgatagaaatatgatccattcatattaggaaaagaaattctggtactgttatttaaataaggcaaaattattccctggattgtttggtgttgtcacctagcagatatacattactcttctgcattgttattggcttgcactttgtgggtatcctatgtaaaaaaaatatatgtatatatatatattgcatatgacaaacttggagattttggttagagctgttaacatctgaattatcaaatgcattacttgtttttgtaaggtactaaatatttaataatacttaaaggaaacccttttgtgtggtccttcggcttacaatgtgcactgaatagttttgtataaggatccagagtggcatttgaaattcgcatgtgctttatattttctatatttgtaactttgcatgtacttgttttattgtattaaaagtttataaatgtttattatctgactaaaattaaaacaggagctacaatgag

SEQ ID NO: 2 - DNA, 514 bp, Sus scrofa
cttggcacaggggccctaggccccataggtgctgatagccctcattatagccccattagcagagctgccagggtccctacaagaaggtgcctggttacaagaattattactttacttatttatgcaccatgtggaagtttccaggctagaagtcgaatcagagatgtagctgctggcctacgccacagccataccagatctgagctgcatctgcgacctcaccacagcacacggcaaggccagggatcgaacccgcgtcctcatggatactaatccatggctggtttctgctgagtcatgatgggaactcccagaatcacaaaagctcaaagctgtggcaaacccaccaggtgtttattggtttttccagtttagatacaatgtatcaagcagaggttatttttaccataagcatgttgctggcattccacctttatcttttctaagaaacagagccagaaaattatctgaaggtcaaatttgtccttagagaaggagaaagagttgagttaac

SEQ ID NO: 3 - DNA, 1019 bp, Sus scrofa
cggttacatgctggggagtgccatgagcagacccctgatacactttggcagtgactatgaggaccgttactatcgtgaaaacatgtaccgttaccccaaccaagtgtactacaggccagtggatcagtacagcaaccagaacagttttgtgcatgactgcgtcaacatcaccgtcaagcagcacacagtgaccacgaccaccaagggggagaacttcaccgagacggacgtcaagatgatagagcgcgtggtggaacagatgtgcatcacccagtaccagaaagagtacgaggcgtacgcccaaagaggggccagtgtgatcctcttctcctcccctcctgtgatcctcctcatctctttcctccttttcctcatagtgggctgagggtggcctttctgtcggcatcatcttcttaatctttatcaggttgggggagggaatatctacctgcagccctttagtggtggtgtctcattcttgcttctctcttcggcacccataggctaacatccatggcgcttgtagcactggaaaaggagagtagacctgagatgtgatgtatttaagccccatttgattgaatccttcataggccagtgctagtgctggactggtaagagcgtaacagcaaataatcattggttgatctgggctcattttttgtctggtgcaacagattgaggctaaaacaattctcaaaacacacttcaagtacctttacctaaatacctccagctccttctccagctagagctcagtacacaaatgccccgccatagtagtgattttgtagcaactttcccatttaagaaaacctgactacattttcctgttcaaatagcatttctactgagttggggaggaggccacataatactcattcaaaaaaatgaaactggaaatccttagctcctgggcccagggtcagcccagtggaaagcatgtgtcctgtgtctgcagagaactaaggatattttgcaatttgcagtacaggttacacagcagctattgcatcaag

SEQ ID NO: 4 - DNA, 720 bp, Sus scrofa
atggtgagcaagggcgaggagctgttcaccggggtggtgcccatcctggtcgagctggacggcgacgtgaacggccacaagttcagcgtgtccggcgagggcgagggcgatgccacctacggcaagctgaccctgaagttcatctgcaccaccggcaagctgcccgtgccctggcccaccctcgtgaccaccctgacctacggcgtgcagtgcttcagccgctaccccgaccacatgaagcagcacgacttcttcaagtccgccatgcccgaaggctacgtccaggagcgcaccatcttcttcaaggacgacggcaactacaagacccgcgccgaggtgaagttcgagggcgacaccctggtgaaccgcatcgagctgaagggcatcgacttcaaggaggacggcaacatcctggggcacaagctggagtacaactacaacagccacaacgtctatatcatggccgacaagcagaagaacggcatcaaggtgaacttcaagatccgccacaacatcgaggacggcagcgtgcagctcgccgaccactaccagcagaacacccccatcggcgacggccccgtgctgctgcccgacaaccactacctgagcacccagtccgccctgagcaaagaccccaacgagaagcgcgatcacatggtcctgctggagttcgtgaccgccgccgggatcactcacggcatggacgagctgtacaagtaa

SEQ ID NO: 5 - DNA, 29 bp, Sus scrofa
ctagacgcgtcttggcacaggggccctag

SEQ ID NO: 6 - DNA, 30 bp, Sus scrofa
gactacgtacgcctaccactgccccagctg

SEQ ID NO: 7 - DNA, 29 bp, Sus scrofa
gactctcgagcggttacatgctggggagt

SEQ ID NO: 8 - DNA, 31 bp, Sus scrofa
gtcaggcgcgccttgatgcaatagctgctgt

SEQ ID NO: 9 - DNA, 20 bp, Sus scrofa
ccagctggggctcgactaga

SEQ ID NO: 10 - DNA, 22 bp, Sus scrofa
ccattttgagcagcctcatttg

SEQ ID NO: 11 - DNA, 34 bp, Sus scrofa
ataacttcgtataatgtatgctatacgaacggta

SEQ ID NO: 12 - DNA, 184 bp, Sus scrofa
ggtggcagaaggagtggataaagaggcaaaattgcctgccaaaaagaaaagaaagaagggtttgcgaattctaccgttcgtatagcatacattatacgaagttataggggaaaaggcgacgaaagaaactgatccttgcaaaaaagtttagtaaggatttgggatctgggaggcctgttgcaag

SEQ ID NO: 13 - DNA, 67 bp, Sus scrofa
agaagggtttgcgaattctaccgttcgtatagcatacattatacgaagttataggggaaaaggcgac

SEQ ID NO: 14 - DNA, 71 bp, Sus scrofa
ggtggcagaaggagtggataaagaggcaaaattgcctgccaaaaagaaaagaaagaagggtttgcgaattc

SEQ ID NO: 15 - DNA, 79 bp, Sus scrofa
aggggaaaaggcgacgaaagaaactgatccttgcaaaaaagtttagtaaggatttgggatctgggaggcctgttgcaag

SEQ ID NO: 16 - DNA, 65 bp, Sus scrofa
agaagggtttgcgaatcctaccgttcgtatgcatacattatacgaagttaaggggaaaaggcgac

SEQ ID NO: 17 - DNA, 65 bp, Sus scrofa
agaagggtttgcgaattctaccgttcgtatgcatacattatacgaagttaaggggaaaaggcggc